European Patent Application EP 4 640 694 A1, published October 29, 2025. Title: SELF-ASSEMBLING PEPTIDE. Applicant: 矩阵（天津）生物科技有限公司. The sequence listing filed with the application follows.

SEQUENCE LISTING (102 sequences)

SEQ ID NO: 1 - protein, 19 aa, synthetic construct
IIIIIGSIIGPGGDGPGGV

SEQ ID NO: 2 - protein, 19 aa, synthetic construct
IIIIIGSIIGPGGEGPGGV

SEQ ID NO: 3 - protein, 19 aa, synthetic construct
IIIIIGSIIGOGGEGPGGV

SEQ ID NO: 4 - protein, 18 aa, synthetic construct
IIIIGSIIGOGGEGPGGV

SEQ ID NO: 5 - protein, 20 aa, synthetic construct
IIIIIGSIIGOGGEGPGGGV

SEQ ID NO: 6 - protein, 18 aa, synthetic construct
IIIIIGSIIGOGGEGPGV

SEQ ID NO: 7 - protein, 19 aa, synthetic construct
IIIIIGSIIGOGAEGPGGV

SEQ ID NO: 8 - protein, 19 aa, synthetic construct
IIIIIGSIIOGGAEGPGGV

SEQ ID NO: 9 - protein, 19 aa, synthetic construct
IIIIIGSIIGOGGVGPGGV

SEQ ID NO: 10 - protein, 25 aa, synthetic construct
IIIIIIGSIIGOGAEGPGGVGPGGV

SEQ ID NO: 11 - protein, 19 aa, synthetic construct
FLIVIGSIIGOGGEGPGGV

SEQ ID NO: 12 - protein, 19 aa, synthetic construct
FLIIAGSIIGPGGDGOGGV

SEQ ID NO: 13 - protein, 20 aa, synthetic construct
IIIIIGOGIIGPGGEGPGGE

SEQ ID NO: 14 - protein, 19 aa, synthetic construct
FIFIFGTVIGPGGEGOGGV

SEQ ID NO: 15 - protein, 19 aa, synthetic construct
IFIFIGTVIGPGGEGOGGK

SEQ ID NO: 16 - protein, 19 aa, synthetic construct
IAILIGTVIGPGGEGOGGE

SEQ ID NO: 17 - protein, 19 aa, synthetic construct
IVIVIGSIIGPGGDGPGGV

SEQ ID NO: 18 - protein, 19 aa, synthetic construct
IVIVIGSIIGOGGDGPGGV

SEQ ID NO: 19 - protein, 19 aa, synthetic construct
IVIVIGSIIGPGGEGOGGV

SEQ ID NO: 20 - protein, 20 aa, synthetic construct
FLIVIGOGIIGOGGEGPGGE

SEQ ID NO: 21 - protein, 20 aa, synthetic construct
IVIVIGOGIIGOGGDGOGGV

SEQ ID NO: 22 - protein, 20 aa, synthetic construct
IVIVIGSGIIGPGGEGPGGV

SEQ ID NO: 23 - protein, 19 aa, synthetic construct
FIIIVGSIIGPGGEGPGGV

SEQ ID NO: 24 - protein, 19 aa, synthetic construct
FIIIVGSIIGPGGEGPGGE

SEQ ID NO: 25 - protein, 20 aa, synthetic construct
IIIIIGOGIIGOGGEGPGGV

SEQ ID NO: 26 - protein, 19 aa, synthetic construct
  MOD_RES 1: note = Acetylation
IIIIIGSIIGPGGEGOGGV

SEQ ID NO: 27 - protein, 19 aa, synthetic construct
FLIVIGSIIGOGAEGPGGV

SEQ ID NO: 28 - protein, 19 aa, synthetic construct
FLIVIGSIIGOGAEGOGGV

SEQ ID NO: 29 - protein, 19 aa, synthetic construct
LLLLLGSVLGPAGEGPAGE

SEQ ID NO: 30 - protein, 20 aa, synthetic construct
LLLLLGPOGLGPAGEGPAGE

SEQ ID NO: 31 - protein, 20 aa, synthetic construct
LLLLLGPOGVGPAGEGPAGE

SEQ ID NO: 32 - protein, 20 aa, synthetic construct
LLLLLGPOGIGPAGEGPAGE

SEQ ID NO: 33 - protein, 4 aa, synthetic construct
GPGG

SEQ ID NO: 34 - protein, 4 aa, synthetic construct
GPGA

SEQ ID NO: 35 - protein, 4 aa, synthetic construct
GPAG

SEQ ID NO: 36 - protein, 4 aa, synthetic construct
GPAA

SEQ ID NO: 37 - protein, 5 aa, synthetic construct
GPGGG

SEQ ID NO: 38 - protein, 4 aa, synthetic construct
GOGG

SEQ ID NO: 39 - protein, 4 aa, synthetic construct
GOGA

SEQ ID NO: 40 - protein, 4 aa, synthetic construct
GOAG

SEQ ID NO: 41 - protein, 5 aa, synthetic construct
GOGGA

SEQ ID NO: 42 - protein, 4 aa, synthetic construct
GOAA

SEQ ID NO: 43 - protein, 4 aa, synthetic construct
GOGV

SEQ ID NO: 44 - protein, 5 aa, synthetic construct
GPAGE

SEQ ID NO: 45 - protein, 5 aa, synthetic construct
GPGGE

SEQ ID NO: 46 - protein, 5 aa, synthetic construct
GOGAE

SEQ ID NO: 47 - protein, 6 aa, synthetic construct
GOGGAE

SEQ ID NO: 48 - protein, 4 aa, synthetic construct
GOGE

SEQ ID NO: 49 - protein, 5 aa, synthetic construct
GOGGE

SEQ ID NO: 50 - protein, 5 aa, synthetic construct
GPGAD

SEQ ID NO: 51 - protein, 5 aa, synthetic construct
GOGGD

SEQ ID NO: 52 - protein, 5 aa, synthetic construct
GPGGV

SEQ ID NO: 53 - protein, 5 aa, synthetic construct
GOGGV

SEQ ID NO: 54 - protein, 5 aa, synthetic construct
GPGGK

SEQ ID NO: 55 - protein, 5 aa, synthetic construct
GOGGK

SEQ ID NO: 56 - protein, 5 aa, synthetic construct
GPGAE

SEQ ID NO: 57 - protein, 5 aa, synthetic construct
GOGAD

SEQ ID NO: 58 - protein, 5 aa, synthetic construct
GPAAD

SEQ ID NO: 59 - protein, 5 aa, synthetic construct
GOAAE

SEQ ID NO: 60 - protein, 5 aa, synthetic construct
GPGGD

SEQ ID NO: 61 - protein, 6 aa, synthetic construct
GPGGGV

SEQ ID NO: 62 - protein, 4 aa, synthetic construct
GPGV

SEQ ID NO: 63 - protein, 5 aa, synthetic construct
GOGGI

SEQ ID NO: 64 - protein, 5 aa, synthetic construct
GOGVI

SEQ ID NO: 65 - protein, 4 aa, synthetic construct
LLLL

SEQ ID NO: 66 - protein, 5 aa, synthetic construct
FIIII

SEQ ID NO: 67 - protein, 5 aa, synthetic construct
IIIII

SEQ ID NO: 68 - protein, 4 aa, synthetic construct
IIII

SEQ ID NO: 69 - protein, 5 aa, synthetic construct
ILILI

SEQ ID NO: 70 - protein, 5 aa, synthetic construct
FLFLF

SEQ ID NO: 71 - protein, 5 aa, synthetic construct
IVIVI

SEQ ID NO: 72 - protein, 6 aa, synthetic construct
VLFIIV

SEQ ID NO: 73 - protein, 5 aa, synthetic construct
VLIII

SEQ ID NO: 74 - protein, 5 aa, synthetic construct
IVALF

SEQ ID NO: 75 - protein, 5 aa, synthetic construct
LFIVL

SEQ ID NO: 76 - protein, 5 aa, synthetic construct
FIAIV

SEQ ID NO: 77 - protein, 5 aa, synthetic construct
FIIIV

SEQ ID NO: 78 - protein, 6 aa, synthetic construct
  MOD_RES 1: note = Acetylation
VLFIIV

SEQ ID NO: 79 - protein, 5 aa, synthetic construct
  MOD_RES 1: note = Acetylation
IVIVI

SEQ ID NO: 80 - protein, 5 aa, synthetic construct
  MOD_RES 1: note = Acetylation
IIIII

SEQ ID NO: 81 - protein, 6 aa, synthetic construct
IIIIII

SEQ ID NO: 82 - protein, 5 aa, synthetic construct
FLIVI

SEQ ID NO: 83 - protein, 5 aa, synthetic construct
FLIIA

SEQ ID NO: 84 - protein, 5 aa, synthetic construct
FIFIF

SEQ ID NO: 85 - protein, 5 aa, synthetic construct
IFIFI

SEQ ID NO: 86 - protein, 5 aa, synthetic construct
IAILI

SEQ ID NO: 87 - protein, 5 aa, synthetic construct
LLLLL

SEQ ID NO: 88 - protein, 5 aa, synthetic construct
GPOGI

SEQ ID NO: 89 - protein, 5 aa, synthetic construct
GPOGV

SEQ ID NO: 90 - protein, 5 aa, synthetic construct
GPOGL

SEQ ID NO: 91 - protein, 4 aa, synthetic construct
GSII

SEQ ID NO: 92 - protein, 5 aa, synthetic construct
GSGII

SEQ ID NO: 93 - protein, 4 aa, synthetic construct
GSVI

SEQ ID NO: 94 - protein, 4 aa, synthetic construct
GOII

SEQ ID NO: 95 - protein, 4 aa, synthetic construct
OGII

SEQ ID NO: 96 - protein, 4 aa, synthetic construct
GTVI

SEQ ID NO: 97 - protein, 4 aa, synthetic construct
GSVL

SEQ ID NO: 98 - protein, 4 aa, synthetic construct
GTII

SEQ ID NO: 99 - protein, 4 aa, synthetic construct
GOVI

SEQ ID NO: 100 - protein, 5 aa, synthetic construct
GSGVI

SEQ ID NO: 101 - protein, 5 aa, synthetic construct
GOGVI

SEQ ID NO: 102 - protein, 5 aa, synthetic construct
GOGII